European Patent Specification EP 4 384 019 B1, published June 25, 2025. Title: Verfahren zum Entfernen von Acrylamid aus Lebens- und Genussmitteln. Applicant: ANKA Angewandte Kaffeetechnologie GmbH. Application WO. The sequence listing filed with the application follows.

SEQUENCE LISTING (44 sequences)

SEQ ID NO: 1 - protein, 513 aa, synthetic construct
  REGION 1..513: note = Artificial Seqence
MSIHMPDPDAVARMAAEGRFGIPESDLPTYHASVTGLLGSWNKVEELYAEVAPTPPQRSWTRPDAEDNKLGAWAVQTSITETSEGPLAGRTVAVKDNVAVAGVPMMNGSRTLEGFVPAEDATVVSRLLAAGATIAGKSVCEDLCFSGGSHTSKPGPVHNPWDMSRSAGGSSSGSGALVAAGEVDMAIGGDQGGSIRIPSAYCGTVGHKPTHGLVPYTGGFPIEQSIDHLGPITRTVADAALMLSVIAGRDGLDPRQPDVVEVQDYVGALAESVSGLRIGVLQEGFGHPNSEPEVDDTVRAAVGTLREAGFTVEDVSVPWHLHATAIWDVIATEGGLWQMVEGNAYGMNWKGHYDPSLIAYYGRKWREDPAQFSETVKLVALAGRYALTTQYGRHYAMARNLAPKLVAAYDAALSNYDVLVMPTLPMRATVLPGPDAPVEEILARGLEMLANTAPFDVTGHPACSVPAGLADGLPVGLMIVGKHFDDATVLKVANAFEQAVGGFPTPAAERSSA

SEQ ID NO: 2 - protein, 513 aa, synthetic construct
  REGION 1..513: note = Artificial Sequence
MSIHMPDPDAVARMAAEGRFGIPESDLPTYHASVTGLLGSWNKVEELYAEVAPTPPQRSWTRPDAEDDKLGAWYVQTSITETSEGPLAGRTVAVKDNVAVAGVPMMNGSRTLEGFVPAEDATVVSRLLAAGATIAGKSVCEDLCFSGGSHTSKPGPVHNPWDMSRSAGGSSSGSGALVAAGEVDMAIGGDQGGSIRIPSAYCGTVGHKPTHGLVPYTGGFPIEQSIDHLGPITRTVADAALMLSVIAGRDGLDPRQPDVVEVQDYVGALAESVSGLRIGVLQEGFGHPNSEPEVDDTVRAAVGTLREAGFTVEDVSVPWHLHATAIWDVIATEGGLWQMVEGNAYGMNWKGHYDPSLIAYYGRKWREDPAQFSETVKLVALAGRYALTTQYGRHYAMARNLAPKLVAAYDAALSNYDVLVMPTLPMRATVLPGPDAPVEEILARGLEMLANTAPFDVTGHPACSVPAGLADGLPVGLMIVGKHFDDATVLKVANAFEQAVGGFPTPAAERSSA

SEQ ID NO: 3 - protein, 513 aa, synthetic construct
  REGION 1..513: note = Artificial Sequence
MSIHMPDPDAVARMAAEGRFGIPESDLPTYHASVTGLLGSWNKVEELYAEVAPTPPQRSWTRPDAEDDKLGAWAVQTSITETSEGPLAGRTVAVKDNVAVAGVPMMNGSRTLEGFVPAEDATVVSRLLAAGATIAGKSVCEDLCFSGGSHTSKPGPVHNPWDMSRSAGGSSSGSGALVAAGEVDMAIGGDQGGSIRIPSAYCGTVGHKPTHGLVPYTGGFPIEQSIDHLGPITRTVADAALMLSVIAGRDGLDPRQPDVVEVQDYVGALAESVSGLRIGVLQEGFGHPNSEPEVDDTVRAAVGTLREAGFTVEDVSVPWHLHATAIWDVIATEGGLWQMVEGNAYGMNWKGHYDPSLIAYYGRKWREDPAQFSETVKLVALAGRYALTTQYGRHYAMARNLAPKLVAAYDAALSNYDVLVMPTLPMRATVLPGPDAPVEEILARALEMLANTAPFDVTGHPACSVPAGLADGLPVGLMIVGKHFDDATVLKVANAFEQAVGGFPTPAAERSSA

SEQ ID NO: 4 - protein, 513 aa, synthetic construct
  REGION 1..513: note = Artificial Sequence
MSIHMPDPDAVARMAAEGRFGIPESDLPTYHAFVTGLLGSWNKVEELYAEVAPTPPQRSWTRPDAEDDKLGAWAVQTSITETSEGPLAGRTVAVKDNVAVAGVPMMNGSRTLEGFVPAEDATVVSRLLAAGATIAGKSVCEDLCFSGGSHTSKPGPVHNPWDMSRSAGGSSSGSGALVAAGEVDMAIGGDQGGSIRIPSAYCGTVGHKPTHGLVPYTGGFPIEQSIDHLGPITRTVADAALMLSVIAGRDGLDPRQPDVVEVQDYVGALAESVSGLRIGVLQEGFGHPNSEPEVDDTVRAAVGTLREAGFTVEDVSVPWHLHATAIWDVIATEGGLWQMVEGNAYGMNWKGHYDPSLIAYYGRKWREDPAQFSETVKLVALAGRYALTTQYGRHYAMARNLAPKLVAAYDAALSNYDVLVMPTLPMRATVLPGPDAPVEEILARGLEMLANTAPFDVTGHPACSVPAGLADGLPVGLMIVGKHFDDATVLKVANAFEQAVGGFPTPAAERSSA

SEQ ID NO: 5 - protein, 513 aa, synthetic construct
  REGION 1..513: note = Artificial Sequence
MSIHMPDPDAVARMAAEGRFGIPESDLPTYHARVTGLLGSWNKVEELYAEVAPTPPQRSWTRPDAEDDKLGAWAVQTSITETSEGPLAGRTVAVKDNVAVAGVPMMNGSRTLEGFVPAEDATVVSRLLAAGATIAGKSVCEDLCFSGGSHTSKPGPVHNPWDMSRSAGGSSSGSGALVAAGEVDMAIGGDQGGSIRIPSAYCGTVGHKPTHGLVPYTGGFPIEQSIDHLGPITRTVADAALMLSVIAGRDGLDPRQPDVVEVQDYVGALAESVSGLRIGVLQEGFGHPNSEPEVDDTVRAAVGTLREAGFTVEDVSVPWHLHATAIWDVIATEGGLWQMVEGNAYGMNWKGHYDPSLIAYYGRKWREDPAQFSETVKLVALAGRYALTTQYGRHYAMARNLAPKLVAAYDAALSNYDVLVMPTLPMRATVLPGPDAPVEEILARGLEMLANTAPFDVTGHPACSVPAGLADGLPVGLMIVGKHFDDATVLKVANAFEQAVGGFPTPAAERSSA

SEQ ID NO: 6 - protein, 513 aa, synthetic construct
  REGION 1..513: note = Artificial squence
MSIHMPDPDAVARMAAEGRFGIPESDLPTYHASVTGLLGSWNKVEELYAEVAPTPPQRSWTRPDAEDDKLGAWAVQTSITETSEGPLAGRTVAVKDNVAVAGVPMMNGSRTLEGFVPAEDATVVSRLLAAGATIAGKSVCEDLCFSGGSHTSKPGPVHNPWDMSRSAGGSSSGSGALVAAGEVDMAIGGDQGGSIRIPSAYCGTVGHKPTHGLVPYTGGFPIEQSIDHLGPITRTVADAALMLSVIAGRDGLDPRQPDVVEVQDYVGALAESVSGLRIGVLQEGFGHPNSEPEVDDTVRAAVGTLREAGFTVEDVSVPWHLHATAIWDVIATEGGLWQMVEGNAYGMNWKGHYDPSLIAYYGRKWREDPAQFSETVKLVALAGRYALTTQYGRHYAMARNLAPKLVAAYDAALSNYDVLVMPTLPMRATVLPGPDAPVEEILARSLEMLANTAPFDVTGHPACSVPAGLADGLPVGLMIVGKHFDDATVLKVANAFEQAVGGFPTPAAERSSA

SEQ ID NO: 7 - protein, 513 aa, synthetic construct
  REGION 1..513: note = Artificial Sequence
MSIHMPDPDAVARMAAEGRFGIPESDLPTYHARVTGLLGSWNKVEELYAEVAPTPPQRSWTRPDAEDDKLGAWYVQTSITETSEGPLAGRTVAVKDNVAVAGVPMMNGSRTLEGFVPAEDATVVSRLLAAGATIAGKSVCEDLCFSGGSHTSKPGPVHNPWDMSRSAGGSSSGSGALVAAGEVDMAIGGDQGGSIRIPSAYCGTVGHKPTHGLVPYTGGFPIEQTIDHLGPITRTVADAALMLSVIAGRDGLDPRQPDVVEVQDYVGALAESVSGLRIGVLQEGFGHPNSEPEVDDTVRAAVGTLREAGFTVEDVSVPWHLHATAIWDVIATEGGLWQMVEGNAYGMNWKGHYDPSLIAYYGRKWREDPAQFSETVKLVALAGRYALTTQYGRHYAMARNLAPKLVAAYDAALSNYDVLVMPTLPMRATVLPGPDAPVEEILARSLEMLANTCPFDVTGHPACSVPAGLADGLPVGLMIVGKHFDDATVLKVANAFEQAVGGFPTPAAERSSA

SEQ ID NO: 8 - protein, 513 aa, synthetic construct
  REGION 1..513: note = Artificial sequence
MSIHMPDPDAVARMAAEGRFGIPESDLPTYHARVTGLLGSWNKVEELYAEVAPTPPQRSWTRPDAEDNKLGAWYVQTSITETSEGPLAGRTVAVKDNVAVAGVPMMNGSRTLEGFVPAEDATVVSRLLAAGATIAGKSVCEDLCFSGGSHTSKPGPVHNPWDMSRSAGGSSSGSGALVAAGEVDMAIGGDQGGSIRIPSAYCGTVGHKPTHGLVPYTGGFPIEQTIDHLGPITRTVADAALMLSVIAGRDGLDPRQPDVVEVQDYVGALAESVSGLRIGVLQEGFGHPNSEPEVDDTVRAAVGTLREAGFTVEDVSVPWHLHATAIWDVIATEGGLWQMVEGNAYGMNWKGHYDPSLIAYYGRKWREDPAQFSETVKLVALAGRYALTTQYGRHYAMARNLAPKLVAAYDAALSNYDVLVMPTLPMRATVLPGPDAPVEEILARSLEMLANTCPFDVTGHPACSVPAGLADGLPVGLMIVGKHFDDATVLKVANAFEQAVGGFPTPAAERSSA

SEQ ID NO: 9 - protein, 513 aa, synthetic construct
  REGION 1..513: note = Artificial sequence
MSIHMPDPDAVARMAAEGRFGIPESDLPTYHARVTGLLGSWNKVEELYAEVAPTPPQRSWTRPDAEDNKLGAWYVQTSITETSEGPLAGRTVAVKDNVAVAGVPMMNGSRTLEGFVPAEDATVVSRLLAAGATIAGKSVCEDLCFSGGSHTSKPGPVHNPWDMSRSAGGSSSGSGALVAAGEVDMAIGGDQGGSIRIPSAYCGTVGHKPTHGLVPYTGGFPIEQTIDHLGPITRTVADAALMLSVIAGRDGLDPRQPDVVEVQDYVGALAESVSGLRIGVLQEGFGHPNSEPEVDDTVRAAVGTLREAGFTVEDVSVPWHLHATAIWDVIATEGGLWQMVEGNAYGMNWKGHYDPSLIAYYGRKWREDPAQFSETVKLVALAGRYALTTQYGRHYAMARNLAPKLVAAYDAALSNYDVLVMPTLPMRATVLPGPDAPVEEILARALEMLANTAPFDVTGHPACSVPAGLADGLPVGLMIVGKHFDDATVLKVANAFEQAVGGFPTPAAERSSA

SEQ ID NO: 10 - protein, 513 aa, synthetic construct
  REGION 1..513: note = Artificial Sequence
MSIHMPDPDAVARMAAEGRFGIPESDLPTYHASVTGLLGSWNKVEELYAEVAPTPPQRSWTRPDAEDNKLGAWYVQTSITETSEGPLAGRTVAVKDNVAVAGVPMMNGSRTLEGFVPAEDATVVSRLLAAGATIAGKSVCEDLCFSGGSHTSKPGPVHNPWDMSRSAGGSSSGSGALVAAGEVDMAIGGDQGGSIRIPSAYCGTVGHKPTHGLVPYTGGFPIEQSIDHLGPITRTVADAALMLSVIAGRDGLDPRQPDVVEVQDYVGALAESVSGLRIGVLQEGFGHPNSEPEVDDTVRAAVGTLREAGFTVEDVSVPWHLHATAIWDVIATEGGLWQMVEGNAYGMNWKGHYDPSLIAYYGRKWREDPAQFSETVKLVALAGRYALTTQYGRHYAMARNLAPKLVAAYDAALSNYDVLVMPTLPMRATVLPGPDAPVEEILARSLEMLANTCPFDVTGHPACSVPAGLADGLPVGLMIVGKHFDDATVLKVANAFEQAVGGFPTPAAERSSA

SEQ ID NO: 11 - protein, 513 aa, synthetic construct
  REGION 1..513: note = Artificial sequence
MSIHMPDPDAVARMAAEGRFGIPESDLPTYHAHVTGLLGSWNKVEELYAEVAPTPPQRSWTRPDAEDNKLGAWYVQTSITETSEGPLAGRTVAVKDNVAVAGVPMMNGSRTLEGFVPAEDATVVSRLLAAGATIAGKSVCEDLCFSGGSHTSKPGPVHNPWDMSRSAGGSSSGSGALVAAGEVDMAIGGDQGGSIRIPSAYCGTVGHKPTHGLVPYTGGFPIEQTIDHLGPITRTVADAALMLSVIAGRDGLDPRQPDVVEVQDYVGALAESVSGLRIGVLQEGFGHPNSEPEVDDTVRAAVGTLREAGFTVEDVSVPWHLHATAIWDVIATEGGLWQMVEGNAYGMNWKGHYDPSLIAYYGRKWREDPAQFSETVKLVALAGRYALTTQYGRHYAMARNLAPKLVAAYDAALSNYDVLVMPTLPMRATVLPGPDAPVEEILARGLEMLANTAPFDVTGHPACSVPAGLADGLPVGLMIVGKHFDDATVLKVANAFEQAVGGFPTPAAERSSA

SEQ ID NO: 12 - protein, 513 aa, synthetic construct
  REGION 1..513: note = Artificial Sequence
MSIHMPDPDAVARMAAEGRFGIPESDLPTYHARVTGLLGSYNKVEELYAEVAPTPPQRSWTRPDAEDNKLGAWYVQTSITETSEGPLAGRTVAIKDNVAVAGVPMMNGSRTLEGFVPAEDATVVSRLLAAGATIAGKSVCEDLCFSGGSHTSKPGPVHNPWDMSRSAGGSSSGSGALVAAGEVDMAIGGDQGGSIRIPSAFCGTVGHKPTHGLVPYTGGFPIEQTIDHLGPITRTVADAALMLSVIAGRDGLDPRQPDVVEVQDYVGALAESVSGLRIGVLQEGFGHPNSEPEVDDTVRAAVGTLREAGFTVEDVSVPWHLHATAIWDVIATEGGLWQMVEGNAYGMNWKGHYDPSLIAYYGRKWREDPAQFSETVKLVALAGRYALTTQYGRHYAMARNLAPKLVAAYDAALSNYDVLVMPTVPMRATVLPGPDAPVEEILARALEHLANTDPFDVTGHPACSVPAGLADGLPVGLMIVGKHFDDATVLKVANAFEQAVGGFPTPPAERSSA

SEQ ID NO: 13 - protein, 513 aa, synthetic construct
  REGION 1..513: note = Artificial Sequence
MSIHMPDPDAVARMAAEGRFGIPESDLPTYHARVTGLLGSWNKVEELYAEVAPTPPQRSWTRPDAEDNKLGAWYVQTSITETSEGPLAGRTVAIKDNVAVAGVPMMNGSRTLEGFVPAEDATVVSRLLAAGATIAGKSVCEDLCFSGGSHTSKPGPVHNPWDMSRSAGGSSSGSGALVAAGEVDMAIGGDQGGSIRIPSAFCGTVGHKPTHGLVPYTGGFPIEQTIDHLGPITRTVADAALMLSVIAGRDGLDPRQPDVVEVQDYVGALAESVSGLRIGVLQEGFGHPNSEPEVDDTVRAAVGTLREAGFTVEDVSVPWHLHATAIWDVIATEGGLWQMVEGNAYGMNWKGHYDPSLIAYYGRKWREDPAQFSETVKLVALAGRYALTTQYGRHYAMARNLAPKLVAAYDAALSNYDVLVMPTVPMRATVLPGPDAPVEEILARALEHLANTDPFDVTGHPACSVPAGLADGLPVGLMIVGKHFDDATVLKVANAFEQAVGGFPTPPAERSSA

SEQ ID NO: 14 - protein, 513 aa, synthetic construct
  REGION 1..513: note = Artificial sequence
MSIHMPDPDAVARMAAEGRFGIPESDLPTYHAYVTGLLGSYNKVEELYAEVAPTPPQRSWTRPDAEDNKLGAWYVQTSITETSEGPLAGRTVAIKDNVAVAGVPMMNGSRTLEGFVPAEDATVVSRLLAAGATIAGKSVCEDLCFSGGSHTSKPGPVHNPWDMSRSAGGSSSGSGALVAAGEVDMAIGGDQGGSIRIPSAFCGTVGHKPTHGLVPYTGGFPIEQTIDHLGPITRTVADAALMLSVIAGRDGLDPRQPDVVEVQDYVGALAESVSGLRIGVLQEGFGHPNSEPEVDDTVRAAVGTLREAGFTVEDVSVPWHLHATAIWDVIATEGGLWQMVEGNAYGMNWKGHYDPSLIAYYGRKWREDPAQFSETVKLVALAGRYALTTQYGRHYAMARNLAPKLVAAYDAALSNYDVLVMPTVPMRATVLPGPDAPVEEILARALEHLANTDPFDVTGHPACSVPAGLADGLPVGLMIVGKHFDDATVLKVANAFEQAVGGFPTPAAERSSA

SEQ ID NO: 15 - protein, 513 aa, synthetic construct
  REGION 1..513: note = Artificial Sequence
MSIHMPDPDAVARMAAEGRFGIPESDLPTYHARVTGLLGSYNKVEELYAEVAPTPPQRSWTRPDAEDNKLGAWYVQTSITETSEGPLAGRTVAVKDNVAVAGVPMMNGSRTLEGFVPAEDATVVSRLLAAGATIAGKSVCEDLCFSGGSHTSKPGPVHNPWDMSRSAGGSSSGSGALVAAGEVDMAIGGDQGGSIRIPSAFCGTVGHKPTHGLVPYTGGFPIEQTIDHLGPITRTVADAALMLSVIAGRDGLDPRQPDVVEVQDYVGALAESVSGLRIGVLQEGFGHPNSEPEVDDTVRAAVGTLREAGFTVEDVSVPWHLHATAIWDVIATEGGLWQMVEGNAYGMNWKGHYDPSLIAYYGRKWREDPAQFSETVKLVALAGRYALTTQYGRHYAMARNLAPKLVAAYDAALSNYDVLVMPTVPMRATVLPGPDAPVEEILARALEHLANTAPFDVTGHPACSVPAGLADGLPVGLMIVGKHFDDATVLKVANAFEQAVGGFPTPAAERSSA

SEQ ID NO: 16 - protein, 513 aa, synthetic construct
  REGION 1..513: note = Artificial Sequence
MSIHMPDPDAVARMAAEGRFGIPESDLPTYHARVTGLLGSYNKVEELYAEVAPTPPQRSWTRPDAEDNKLGAWYVQTSITETSEGPLAGRTVAIKDNVAVAGVPMMNGSRTLEGFVPAEDATVVSRLLAAGATIAGKSVCEDLCFSGGSHTSKPGPVHNPWDMSRSAGGSSSGSGALVAAGEVDMAIGGDQGGSIRIPSAFCGTVGHKPTHGLVPYTGGFPIEQTIDHLGPITRTVADAALMLSVIAGRDGLDPRQPDVVEVQDYVGALAESVSGLRIGVLQEGFGHPNSEPEVDDTVRAAVGTLREAGFTVEDVSVPWHLHATAIWDVIATEGGLWQMVEGNAYGMNWKGHYDPSLIAYYGRKWREDPAQFSETVKLVALAGRYALTTQYGRHYAMARNLAPKLVAAYDAALSNYDVLVMPTVPMRATVLPGPDAPVEEILARALEHLANTCPFDVTGHPACSVPAGLADGLPVGLMIVGKHFDDATVLKVANAFEQAVGGFPTPPAERSSA

SEQ ID NO: 17 - protein, 513 aa, synthetic construct
  REGION 1..513: note = Artificial Sequence
MSIHMPDPDAVARMAAEGRFGIPESDLPTYHAYVTGLLGSYNKVEELYAEVAPTPPQRSWTRPDAEDNKLGAWYVQTSITETSEGPLAGRTVAIKDNVAVAGVPMMNGSRTLEGFVPAEDATVVSRLLAAGATIAGKSVCEDLCFSGGSHTSKPGPVHNPWDMSRSAGGSSSGSGALVAAGEVDMAIGGDQGGSIRIPSAFCGTVGHKPTHGLVPYTGGFPIEQTIDHLGPITRTVADAALMLSVIAGRDGLDPRQPDVVEVQDYVGALAESVSGLRIGVLQEGFGHPNSEPEVDDTVRAAVGTLREAGFTVEDVSVPWHLHATAIWDVIATEGGLWQMVEGNAYGMNWKGHYDPSLIAYYGRKWREDPAQFSETVKLVALAGRYALTTQYGRHYAMARNLAPKLVAAYDAALSNYDVLVMPTVPMRATVLPGPDAPVEEILARALEHLANTNPFDVTGHPACSVPAGLADGLPVGLMIVGKHFDDATVLKVANAFEQAVGGFPTPAAERSSA

SEQ ID NO: 18 - protein, 513 aa, synthetic construct
  REGION 1..513: note = Artificial Sequence
MSIHMPDPDAVARMAAEGRFGIPESDLPTYHAYVTGLLGSYNKVEELYAEVAPTPPQRSWTRPDAEDNKLGAWYVQTSITETSEGPLAGRTVAIKDNVAVAGVPMMNGSRTLEGFVPAEDATVVSRLLAAGATIAGKSVCEDLCFSGGSHTSKPGPVHNPWDMSRSAGGSSSGSGALVAAGEVDMAIGGDQGGSIRIPSAFCGTVGHKPTHGLVPYTGGFPIEQTIDHLGPITRTVADAALMLSVIAGRDGLDPRQPDVVEVQDYVGALAESVSGLRIGVLQEGFGHPNSEPEVDDTVRAAVGTLREAGFTVEDVSVPWHLHATAIWDVIATEGGLWQMVEGNAYGMNWKGHYDPSLIAYYGRKWREDPAQFSETVKLVALAGRYALTTQYGRHYAMARNLAPKLVAAYDAALSNYDVLVMPTVPMRATVLPGPDAPVEEILARALEHLANTQPFDVTGHPACSVPAGLADGLPVGLMIVGKHFDDATVLKVANAFEQAVGGFPTPAAERSSA

SEQ ID NO: 19 - protein, 513 aa, synthetic construct
  REGION 1..513: note = Artificial Sequence
MSIHMPDPDAVARMAAEGRFGIPESDLPTYHAYVTGLLGSYNKVEELYAEVAPTPPQRSWTRPDAEDNKLGAWYVQTSITETSEGPLAGRTVAIKDNVAVAGVPMMNGSRTLEGFVPAEDATVVSRLLAAGATIAGKSVCEDLCFSGGSHTSKPGPVHNPWDMSRSAGGSSSGSGALVAAGEVDMAIGGDQGGSIRIPSAFCGTVGHKPTHGLVPYTGGFPIEQTIDHLGPITRTVADAALMLSVIAGRDGLDPRQPDVVEVQDYVGALAESVSGLRIGVLQEGFGHPNSEPEVDDTVRAAVGTLREAGFTVEDVSVPWHLHATAIWDVIATEGGLWQMVEGNAYGMNWKGHYDPSLIAYYGRKWREDPAQFSETVKLVALAGRYALTTQYGRHYAMARNLAPKLVAAYDAALSNYDVLVMPTVPMRATVLPGPDAPVEEILARALEHLANTEPFDVTGHPACSVPAGLADGLPVGLMIVGKHFDDATVLKVANAFEQAVGGFPTPAAERSSA

SEQ ID NO: 20 - protein, 513 aa, synthetic construct
  REGION 1..513: note = Artificial Sequence
MSIHMPDPDAVARMAAEGRFGIPESDLPTYHAYVTGLLGSYNKVEELYAEVAPTPPQRSWTRPDAEDNKLGAWYVQTSITETSEGPLAGRTVAIKDNVAVAGVPMMNGSRTLEGFVPAEDATVVSRLLAAGATIAGKSVCEDLCFSGGSHTSKPGPVHNPWDMSRSAGGSSSGSGALVAAGEVDMAIGGDQGGSIRIPSAFCGTVGHKPTHGLVPYTGGFPIEQTIDHLGPITRTVADAALMLSVIAGRDGLDPRQPDVVEVQDYVGALAESVSGLRIGVLQEGFGHPNSEPEVDDTVRAAVGTLREAGFTVEDVSVPWHLHATAIWDVIATEGGLWQMVEGNAYGMNWKGHYDPSLIAYYGRKWREDPAQFSETVKLVALAGRYALTTQYGRHYAMARNLAPKLVAAYDAALSNYDVLVMPTVPMRATVLPGPDAPVEEILARALEHLANTKPFDVTGHPACSVPAGLADGLPVGLMIVGKHFDDATVLKVANAFEQAVGGFPTPAAERSSA

SEQ ID NO: 21 - protein, 513 aa, synthetic construct
  REGION 1..513: note = Artificial Sequence
MSIHMPDPDAVARMAAEGRFGIPESDLPTYHARVTGLLGSWNKVEELYAEVAPTPPQRSWTRPDAEDNKLGAWYVQTSITETSEGPLAGRTVAVKDNVAVAGVPMMNGSRTLEGFVPAEDATVVSRLLAAGATIAGKSVCEDLCFSGGSHTSKPGPVHNPWDMSRSAGGSSSGSGALVAAGEVDMAIGGDQGGSIRIPSAYCGTVGHKPTHGLVPYTGGFPIEQTIDHLGPITRTVADAALMLSVIAGRDGLDPRQPDVVEVQDYVGALAESVSGLRIGVLQEGFGHPNSEPEVDDTVRAAVGTLREAGFTVEDVSVPWHLHATAIWDVIATEGGLWQMVEGNAYGMNWKGHYDPSLIAYYGRKWREDPAQFSETVKLVALAGRYALTTQYGRHYAMARNLAPKLVAAYDAALSNYDVLVMPTLPMRATVLPGPDAPVEEILARALEMLANTANFDVTGHPACSVPAGLADGLPVGLMIVGKHFDDATVLKVANAFEQAVGGFPTPAAERSSA

SEQ ID NO: 22 - protein, 1026 aa, synthetic construct
  REGION 1..1026: note = Artificial Sequence
MSIHMPDPDAVARMAAEGRFGIPESDLPTYHARVTGLLGSWNKVEELYAEVAPTPPQRSWTRPDAEDNKLGAWYVQTSITETSEGPLAGRTVAVKDNVAVAGVPMMNGSRTLEGFVPAEDATVVSRLLAAGATIAGKSVCEDLCFSGGSHTSKPGPVHNPWDMSRSAGGSSSGSGALVAAGEVDMAIGGDQGGSIRIPSAYCGTVGHKPTHGLVPYTGGFPIEQTIDHLGPITRTVADAALMLSVIAGRDGLDPRQPDVVEVQDYVGALAESVSGLRIGVLQEGFGHPNSEPEVDDTVRAAVGTLREAGFTVEDVSVPWHLHATAIWDVIATEGGLWQMVEGNAYGMNWKGHYDPSLIAYYGRKWREDPAQFSETVKLVALAGRYALTTQYGRHYAMARNLAPKLVAAYDAALSNYDVLVMPTLPMRATVLPGPDAPVEEILARALEMLANTAPFDGTGHPACSVPAGLADGLPVGLMIVGKHFDDATVLKVANAFEQAVGGFPTPAAERSSAMSIHMPDPDAVARMAAEGRFGIPESDLPTYHARVTGLLGSWNKVEELYAEVAPTPPQRSWTRPDAEDNKLGAWYVQTSITETSEGPLAGRTVAVKDNVAVAGVPMMNGSRTLEGFVPAEDATVVSRLLAAGATIAGKSVCEDLCFSGGSHTSKPGPVHNPWDMSRSAGGSSSGSGALVAAGEVDMAIGGDQGGSIRIPSAYCGTVGHKPTHGLVPYTGGFPIEQTIDHLGPITRTVADAALMLSVIAGRDGLDPRQPDVVEVQDYVGALAESVSGLRIGVLQEGFGHPNSEPEVDDTVRAAVGTLREAGFTVEDVSVPWHLHATAIWDVIATEGGLWQMVEGNAYGMNWKGHYDPSLIAYYGRKWREDPAQFSETVKLVALAGRYALTTQYGRHYAMARNLAPKLVAAYDAALSNYDVLVMPTVPMRATVLPGPDAPVEEILARALEMLANTAPFDVTGHPACSVPAGLADGLPVGLMIVGKHFDDATVLKVANAFEQAVGGFPTPAAERSSA

SEQ ID NO: 23 - protein, 513 aa, synthetic construct
  REGION 1..513: note = Artificial sequence
MSIHMPDPDAVARMAAEGRFGIPESDLPTYHARVTGLLGSWNKVEELYAEVAPTPPQRSWTRPDAEDNKLGAWYVQTSITETSEGPLAGRTVAVKDNVAVAGVPMMNGSRTLEGFVPAEDATVVSRLLAAGATIAGKSVCEDLCFSGGSHTSKPGPVHNPWDMSRSAGGSSSGSGALVAAGEVDMAIGGDQGGSIRIPSAYCGTVGHKPTHGLVPYTGGFPIEQTIDHLGPITRTVADAALMLSVIAGRDGLDPRQPDVVEVQDYVGALAESVSGLRIGVLQEGFGHPNSEPEVDDTVRAAVGTLREAGFTVEDVSVPWHLHATAIWDVIATEGGLWQMVEGNAYGMNWKGHYDPSLIAYYGRKWREDPAQFSETVKLVALAGRYALTTQYGRHYAMARNLAPKLVAAYDAALSNYDVLVMPTVPMRATVLPGPDAPVEEILARALEMLANTAPFDVTGHPACSVPAGLADGLPVGLMIVGKHFDDATVLKVANAFEQAVGGFPTPAAERSSA

SEQ ID NO: 24 - protein, 513 aa, synthetic construct
  REGION 1..513: note = Artificial Sequence
MSIHMPDPDAVARMAAEGRFGIPESDLPTYHARVTGLLGSWNKVEELYAEVAPTPPQRSWTRPDAEDNKLGAWYVQTSITETSEGPLAGRTVAVKDNVAVAGVPMMNGSRTLEGFVPAEDATVVSRLLAAGATIAGKSVCEDLCFSGGSHTSKPGPVHNPWDMSRSAGGSSSGSGALVAAGEVDMAIGGDQGGSIRIPSAYCGTVGHKPTHGLVPYTGGFPIEQTIDHLGPITRTVADAALMLSVIAGRDGLDPRQPDVVEVQDYVGALAESVSGLRIGVLQEGFGHPNSEPEVDDTVRAAVGTLREAGFTVEDVSVPWHLHATAIWDVIATEGGLWQMVEGNAYGMNWKGHYDPSLIAYYGRKWREDPAQFSETVKLVALAGRYALTTQYGRHYAMARNLAPKLVAAYDAALSNYDVLVMPTLPMRATVLPGPDAPVEEILARALEMLANTDPFDVTGHPACSVPAGLADGLPVGLMIVGKHFDDATVLKVANAFEQAVGGFPTPAAERSSA

SEQ ID NO: 25 - protein, 513 aa, synthetic construct
  REGION 1..513: note = Artificial Sequence
MSIHMPDPDAVARMAAEGRFGIPESDLPTYHAYVTGLLGSWNKVEELYAEVAPTPPQRSWTRPDAEDNKLGAWYVQTSITETSEGPLAGRTVAVKDNVAVAGVPMMNGSRTLEGFVPAEDATVVSRLLAAGATIAGKSVCEDLCFSGGSHTSKPGPVHNPWDMSRSAGGSSSGSGALVAAGEVDMAIGGDQGGSIRIPSAYCGTVGHKPTHGLVPYTGGFPIEQTIDHLGPITRTVADAALMLSVIAGRDGLDPRQPDVVEVQDYVGALAESVSGLRIGVLQEGFGHPNSEPEVDDTVRAAVGTLREAGFTVEDVSVPWHLHATAIWDVIATEGGLWQMVEGNAYGMNWKGHYDPSLIAYYGRKWREDPAQFSETVKLVALAGRYALTTQYGRHYAMARNLAPKLVAAYDAALSNYDVLVMPTLPMRATVLPGPDAPVEEILARALEMLANTAPFDVTGHPACSVPAGLADGLPVGLMIVGKHFDDATVLKVANAFEQAVGGFPTPAAERSSA

SEQ ID NO: 26 - protein, 513 aa, synthetic construct
  REGION 1..513: note = Artificial Sequence
MSIHMPDPDAVARMAAEGRFGIPESDLPTYHARVTGLLGSWNKVEELYAEVAPTPPQRSWTRPDAEDNKLGAWYVQTSITETSEGPLAGRTVAVKDNVAVAGVPMMNGSRTLEGFVPAEDATVVSRLLAAGATIAGKSVCEDLCFSGGSHTSKPGPVHNPWDMSRSAGGSSSGSAALVAAGEVDMAIGGDQGGSIRIPSAYCGTVGHKPTHGLVPYTGGFPIEQTIDHLGPITRTVADAALMLSVIAGRDGLDPRQPDVVEVQDYVGALAESVSGLRIGVLQEGFGHPNSEPEVDDTVRAAVGTLREAGFTVEDVSVPWHLHATAIWDVIATEGGLWQMVEGNAYGMNWKGHYDPSLIAYYGRKWREDPAQFSETVKLVALAGRYALTTQYGRHYAMARNLAPKLVAAYDAALSNYDVLVMPTLPMRATVLPGPDAPVEEILARALEMLANTAPFDVTGHPACSVPAGLADGLPVGLMIVGKHFDDATVLKVANAFEQAVGGFPTPAAERSSA

SEQ ID NO: 27 - protein, 513 aa, synthetic construct
  REGION 1..513: note = Artificial Sequence
MSIHMPDPDAVARMAAEGRFGIPESDLPTYHARVTGLLGSWNKVEELYAEVAPTPPQRSWTRPDAEDNKLGAWYVQTSITETSEGPLAGRTVAVKDNVAVAGVPMMNGSRTLEGFVPAEDATVVSRLLAAGATIAGKSVCEDLCFSGGSHTSKPGPVHNPWDMSRSAGGSSSGSGALVAAGEVDMAIGGDQGGSIRIPSAYCGTVGHKPTHGLVPYTGGFPIEQTIDHLGPITRTVADAALMLSVIAGRDGLDPRQPDVVEVQDYVGALAESVSGLRIGVLQEGFGHPNSEPEVDDTVRAAVGTLREAGFTVEDVSVPWHLHATAIWDVIATEGGLWQMVEGNAYGMNWKGHYDPSLIAYYGRKWREDPAQFSETVKLVALAGRYALTTQYGRHYAMARNLAPKLVAAYDAALSNYDVLVMPTLPMRATVLPGPDAPVEEILARALEMLANTAPFDVTGHPACSVPAGLADGLPVGLMIVGKHFDDATVLKVANAFEQAVGGFPTPPAERSSA

SEQ ID NO: 28 - protein, 513 aa, synthetic construct
  REGION 1..513: note = Artificial Sequence
MSIHMPDPDAVARMAAEGRFGIPESDLPTYHARVTGLLGSWNKVEELYAEVAPTPPQRSWTRPDAEDNKLGAWYVQTSITETSEGPLAGRTVAVKDNVAVAGVPMMNGSRTLEGFVPAEDATVVSRLLAAGATIAGKSVCEDLCFSGGSHTSKPGPVHNPWDMSRSAGGSSSGSGALVAAGEVDMAIGGDQGGSIRIPSAYCGTVGHKPTHGLVPYTGGFPIEQTIDHLGPITRTVADAALMLSVIAGRDGLDPRQPDVVEVQDYVGALAESVSGLRIGVLQEGFGHPNSEPEVDDTVRAAVGTLREAGFTVEDVSVPWHLHATAIWDVIATEGGLWQMVEGNAYGMNWKGHYDPSLIAYYGRKWREDPAQFSETVKLVALAGRYALTTQYGRHYAMARNLAPKLVAAYDAALSNYDVLVMPTLPMRATVLPGPDAPVEEILARALEMLANTSPFDVTGHPACSVPAGLADGLPVGLMIVGKHFDDATVLKVANAFEQAVGGFPTPAAERSSA

SEQ ID NO: 29 - protein, 513 aa, synthetic construct
  REGION 1..513: note = Artificial Sequence
MSIHMPDPDAVARMAAEGRFGIPESDLPTYHARVTGLLGSWNKVEELYAEVAPTPPQRSWTRPDAEDNKLGAWYVQTSITETSEGPLAGRTVAIKDNVAVAGVPMMNGSRTLEGFVPAEDATVVSRLLAAGATIAGKSVCEDLCFSGGSHTSKPGPVHNPWDMSRSAGGSSSGSGALVAAGEVDMAIGGDQGGSIRIPSAYCGTVGHKPTHGLVPYTGGFPIEQTIDHLGPITRTVADAALMLSVIAGRDGLDPRQPDVVEVQDYVGALAESVSGLRIGVLQEGFGHPNSEPEVDDTVRAAVGTLREAGFTVEDVSVPWHLHATAIWDVIATEGGLWQMVEGNAYGMNWKGHYDPSLIAYYGRKWREDPAQFSETVKLVALAGRYALTTQYGRHYAMARNLAPKLVAAYDAALSNYDVLVMPTLPMRATVLPGPDAPVEEILARALEMLANTAPFDVTGHPACSVPAGLADGLPVGLMIVGKHFDDATVLKVANAFEQAVGGFPTPAAERSSA

SEQ ID NO: 30 - protein, 513 aa, synthetic construct
  REGION 1..513: note = Artificial Sequence
MSIHMPDPDAVARMAAEGRFGIPESDLPTYHARVTGLLGSWNKVEELYAEVAPTPPQRSWTRPDAEDNKLGAWYVQTSITETSEGPLAGRTVAVKDNVAVAGVPMMNGSRTLEGFVPAEDATVVSRLLAAGATIAGKSVCEDLCFSGGSHTSKPGPVHNPWDMSRSAGGSSSGSGALVAAGEVDMAIGGDQGGSIRIPSAYCGTVGHKPTHGLVPYTGGFPIEQTIDHLGPITRTVADAALMLSVIAGRDGLDPRQPDVVEVQDYVGALAESVSGLRIGVLQEGFGHPNSEPEVDDTVRAAVGTLREAGFTVEDVSIPWHLHATAIWDVIATEGGLWQMVEGNAYGMNWKGHYDPSLIAYYGRKWREDPAQFSETVKLVALAGRYALTTQYGRHYAMARNLAPKLVAAYDAALSNYDVLVMPTLPMRATVLPGPDAPVEEILARALEMLANTAPFDVTGHPACSVPAGLADGLPVGLMIVGKHFDDATVLKVANAFEQAVGGFPTPAAERSSA

SEQ ID NO: 31 - protein, 513 aa, synthetic construct
  REGION 1..513: note = Artificial Sequence
MSIHMPDPDAVARMAAEGRFGIPESDLPTYHARVTGLLGSWNKVEELYAEVAPTPPQRSWTRPDAEDNKLGAWYVQTSITETSEGPLAGRTVAVKDNVAVAGVPMMNGSRTLEGFVPAEDATVVSRLLAAGATIAGKSVCEDLCFSGGSHTSKPGPVHNPWDMSRSAGGSSSGSGALVAAGEVDMAIGGDQGGSIRIPSAFCGTVGHKPTHGLVPYTGGFPIEQTIDHLGPITRTVADAALMLSVIAGRDGLDPRQPDVVEVQDYVGALAESVSGLRIGVLQEGFGHPNSEPEVDDTVRAAVGTLREAGFTVEDVSVPWHLHATAIWDVIATEGGLWQMVEGNAYGMNWKGHYDPSLIAYYGRKWREDPAQFSETVKLVALAGRYALTTQYGRHYAMARNLAPKLVAAYDAALSNYDVLVMPTLPMRATVLPGPDAPVEEILARALEMLANTAPFDVTGHPACSVPAGLADGLPVGLMIVGKHFDDATVLKVANAFEQAVGGFPTPAAERSSA

SEQ ID NO: 32 - protein, 513 aa, synthetic construct
  REGION 1..513: note = Artificial Sequence
MSIHMPDPDAVARMAAEGRFGIPESDLPTYHARVTGLLGSWNKVEELYAEVAPTPPQRSWTRPDAEDNKLGAWYVQTSITETSEGPLAGRTVAVKDNVAVAGVPMMNGSRTLEGFVPAEDATVVSRLLAAGATIAGKSVCEDLCFSGGSHTSKPGPVHNPWDMSRSAGGSSSGSGALVAAGEVDMAIGGDQGGSIRIPSAYCGTVGHKPTHGLVPYTGGFPIEQTIDHLGPITRTVADAALMLSVIAGRDGLDPRQPDVVEVQDYVGALAESVSGLRIGVLQEGFGHPNSEPEVDDTVRAAVGTLREAGFTVEDVSVPWHLHATAIWDVIATEGGLWQMVEGNAYGMNWKGHYDPSLIAYYGRKWREDPAQFSETVKLVALAGRYALTTQYGRHYAMARNLAPKLVAAYDAALSNYDVLVMPTLPMRATVLPGPDAPVEEILARALEHLANTAPFDVTGHPACSVPAGLADGLPVGLMIVGKHFDDATVLKVANAFEQAVGGFPTPAAERSSA

SEQ ID NO: 33 - protein, 513 aa, synthetic construct
  REGION 1..513: note = Artificial Sequence
MSIHMPDPDAVARMAAEGRFGIPESDLPTYHARVTGLLGSWNKVEELYAEVAPTPPQRSWTRPDAEDNKLGAWYVQTSITETSEGPLAGRTVAVKDNVAVAGVPMMNGSRTLEGFVPAEDATVVSRLLAAGATIAGKSVCEDLCFSGGSHTSKPGPVHNPWDMSRSAGGSSSGSGALVAAGEVDMAIGGDQGGSIRIPSAYCGTVGHKPTHGLVPYTGGFPIEQTIDHLGPITRTVADAALMLSVIAGRDGLDPRQPDVVEVQDYVGALAESVSGLRIGVLQEGFGHPNSEPEVDDTVRAAVGTLREAGFTVEDVSVPWHLHATAIWDVIATEGGLWQMVEGNAYGMNWKGHYDPSLIAYYGRKWREDPAQFSETVKLVALAGRYALTTQYGRHYAMARNLAPKLVAAYDAALSNYDVLVMPTLPMRATVLPGPDAPVEEILARALEMLANTRPFDVTGHPACSVPAGLADGLPVGLMIVGKHFDDATVLKVANAFEQAVGGFPTPAAERSSA

SEQ ID NO: 34 - protein, 513 aa, synthetic construct
  REGION 1..513: note = Artificial Sequence
MSIHMPDPDAVARMAAEGRFGIPESDLPTYHARVTGLLGSWNKVEELYAEVAPTPPQRSWTRPDAEDNKLGAWYVQTSITETSEGPLAGRTVAVKDNVAVAGVPMMNGSRTLEGFVPAEDATVVSRLLAAGATIAGKSVCEDLCFSGGSHTSKPGPVHNPWDMSRSAGGSSSGSGALVAAGEVDMAIGGDQGGSIRIPSAYCGTVGHKPTHGLVPYTGGFGIEQTIDHLGPITRTVADAALMLSVIAGRDGLDPRQPDVVEVQDYVGALAESVSGLRIGVLQEGFGHPNSEPEVDDTVRAAVGTLREAGFTVEDVSVPWHLHATAIWDVIATEGGLWQMVEGNAYGMNWKGHYDPSLIAYYGRKWREDPAQFSETVKLVALAGRYALTTQYGRHYAMARNLAPKLVAAYDAALSNYDVLVMPTLPMRATVLPGPDAPVEEILARALEMLANTAPFDVTGHPACSVPAGLADGLPVGLMIVGKHFDDATVLKVANAFEQAVGGFPTPAAERSSA

SEQ ID NO: 35 - protein, 513 aa, synthetic construct
  REGION 1..513: note = Artificial sequence
MSIHMPDPDAVARMAAEGRFGIPESDLPTYHARVTGLLGSWNKVEELYAEVAPTPPQRSWTRPDAEDNKLGAWYVQTSITETSEGPLAGRTVAVKDNVAVAGVPMMNGSRTLEGFVPAEDATVVSRLLAAGATIAGKSVCEDLCFSGGSHTSKPGPVHNPWDMSRSAGGSSSGSGALVAAGEVDMAIGGDQGGSIRIPSAYCGTVGHKPTHGLVPYRGGFPIEQTIDHLGPITRTVADAALMLSVIAGRDGLDPRQPDVVEVQDYVGALAESVSGLRIGVLQEGFGHPNSEPEVDDTVRAAVGTLREAGFTVEDVSVPWHLHATAIWDVIATEGGLWQMVEGNAYGMNWKGHYDPSLIAYYGRKWREDPAQFSETVKLVALAGRYALTTQYGRHYAMARNLAPKLVAAYDAALSNYDVLVMPTLPMRATVLPGPDAPVEEILARALEMLANTAPFDVTGHPACSVPAGLADGLPVGLMIVGKHFDDATVLKVANAFEQAVGGFPTPAAERSSA

SEQ ID NO: 36 - protein, 513 aa, synthetic construct
  REGION 1..513: note = Artificial Sequence
MSIHMPDPDAVARMAAEGRFGIPESDLPTYHARVTGLLGSWNKVEELYAEVAPTPPQRSWTRPDAEDNKLGAWYVQTSITETSEGPLAGRTVAVKDNVAVAGVPMMNGSRTLEGFVPAEDATVVSRLLAAGATIAGKSVCEDLCFSGGSHTSKPGPVHNPWDMSRSAGGSSSGSGALVAAGEVDMAIGGDQGGSIRIPSAYCGTVGHKPTHGLVPYTGGFPIEQTIDHLGPITRTVADAALMLSVIAGRDGLDPRQPDVVEVQDYVGALAESVSGLRIGVLQEGFGHPNSEPEVDDTVRAAVGTLREAGFTVEDVSVPWHLHATAIWRVIATEGGLWQMVEGNAYGMNWKGHYDPSLIAYYGRKWREDPAQFSETVKLVALAGRYALTTQYGRHYAMARNLAPKLVAAYDAALSNYDVLVMPTLPMRATVLPGPDAPVEEILARALEMLANTAPFDVTGHPACSVPAGLADGLPVGLMIVGKHFDDATVLKVANAFEQAVGGFPTPAAERSSA

SEQ ID NO: 37 - protein, 513 aa, synthetic construct
  REGION 1..513: note = Artificial Sequence
MSIHMPDPDAVARMAAEGRFGIPESDLPTYHARVTGLLGSWNKVEELYAEVAPTPPQRSWTRPDAEDNKLGAWYVQTSITETSEGPLAGRTVAVKDNVAVAGVPMMNGSRTLEGFVPAEDATVVSRLLAAGATIAGKSVCEDLCFSGGSHTSKPGPVHNPWDMSRSAGGSSSGSGALVAAGEVDMAIGGDQGGSIRIPSAYCGTVGHKPTHGLVPYTGGFPIEQTIDHLGPITRTVADAALMLSVIAGRDGLDPRQPDVVEVQDYVGALAESVSGLRIGVLQEGFGHPNSEPEVDDTVRAAVGTLREAGFTVEDVSVPWHLHATAIWDVIATEGGLWQMVEGNAYGMNWKGHYDPSLIAYYGRKWREDPAQFSETVKLVALAGRYALTTQYGRHYAMARNLAPKLVAAYDAALSNYDVLVMPTLPMRATVLPGPDAPVEEILARSLEMLANTAPFDVTGHPACSVPAGLADGLPVGLMIVGKHFDDATVLKVANAFEQAVGGFPTPAAERSSA

SEQ ID NO: 38 - protein, 513 aa, synthetic construct
  REGION 1..513: note = Artificial Sequence
MSIHMPDPDAVARMAAEGRFGIPESDLPTYHARVTGLLGSWNKVEELYAEVAPTPPQRSWTRPDAEDNKLGAWYVQTSITETSEGPLAGRTVAVKDNVAVAGVPMMNGSRTLEGFVPAEDATVVSRLLAAGATIAGKSVCEDLCFSGGSHTSKPGPVHNPWDMSRSAGGSSSGSGALVAAGEVDMAIGGDQGGSIRIPSAYCGTVGHKPTHGLVPYTGGFPIEQTIDHCGPITRTVADAALMLSVIAGRDGLDPRQPDVVEVQDYVGALAESVSGLRIGVLQEGFGHPNSEPEVDDTVRAAVGTLREAGFTVEDVSVPWHLHATAIWDVIATEGGLWQMVEGNAYGMNWKGHYDPSLIAYYGRKWREDPAQFSETVKLVALAGRYALTTQYGRHYAMARNLAPKLVAAYDAALSNYDVLVMPTLPMRATVLPGPDAPVEEILARALEMLANTAPFDVTGHPACSVPAGLADGLPVGLMIVGKHFDDATVLKVANAFEQAVGGFPTPAAERSSA

SEQ ID NO: 39 - protein, 513 aa, synthetic construct
  REGION 1..513: note = Artificial Sequence
MSIHMPDPDAVARMAAEGRFGIPESDLPTYHARVTGLLGSYNKVEELYAEVAPTPPQRSWTRPDAEDNKLGAWYVQTSITETSEGPLAGRTVAVKDNVAVAGVPMMNGSRTLEGFVPAEDATVVSRLLAAGATIAGKSVCEDLCFSGGSHTSKPGPVHNPWDMSRSAGGSSSGSGALVAAGEVDMAIGGDQGGSIRIPSAYCGTVGHKPTHGLVPYTGGFPIEQTIDHLGPITRTVADAALMLSVIAGRDGLDPRQPDVVEVQDYVGALAESVSGLRIGVLQEGFGHPNSEPEVDDTVRAAVGTLREAGFTVEDVSVPWHLHATAIWDVIATEGGLWQMVEGNAYGMNWKGHYDPSLIAYYGRKWREDPAQFSETVKLVALAGRYALTTQYGRHYAMARNLAPKLVAAYDAALSNYDVLVMPTLPMRATVLPGPDAPVEEILARALEMLANTAPFDVTGHPACSVPAGLADGLPVGLMIVGKHFDDATVLKVANAFEQAVGGFPTPAAERSSA

SEQ ID NO: 40 - protein, 348 aa, Parageobacillus thermoglucosidadius
MRHGDISSSHDTVGVAVVNYKMPRLHTKKEVIENAKNIANMIVGMKQGLPGMDLVIFPEYSTMGIMYDRKEMFETATTIPGPETEIFAEACRKANTWGVFSLTGEQHEEHPHKNPYNTLVLINNKGEIVQKYRKIIPWCPIEGWYPGDTTYVTEGPKGIKISLIICDDGNYPEIWRDCAMKGAELIVRCQGYMYPAKEQQIMMAKTMAWANNVYVAVANATGFDGVYSYFGHSAIIGFDGRTLGECGEEENGIQYAEISLSQIRDFRKNAQSQNHLFKLLHRGYTGIIXSGEGDKGVAECPFDFYRTWVMDAEKARENVEKITRTTIGTAECPIEGIPHEGKEKEASV

SEQ ID NO: 41 - protein, 348 aa, Geobacillus pallidus RAPc8
MRHGDISSSHDTVGIAVVNYKMPRLHTKAEVIENAKKIADMVVGMKQGLPGMDLVVFPEYSTMGIMYDQDEMFATAASIPGEETAIFAEACKKADTWGVFSLTGEKHEDHPNKAPYNTLVLINNKGEIVQKYRKIIPWCPIEGWYPGDTTYVTEGPKGLKISLIVCDDGNYPEIWRDCAMKGAELIVRCQGYMYPAKEQQIMMAKAMAWANNTYVAVANATGFDGVYSYFGHSAIIGFDGRTLGECGTEENGIQYAEVSISQIRDFRKNAQSQNHLFKLLHRGYTGLINSGEGDRGVAECPFDFYRTWVLDAEKARENVEKITRSTVGTAECPIQGIPNEGKTKEIGV

SEQ ID NO: 42 - protein, 348 aa, Geobacillus stearothermophilus
MRHGDISSSHDTVGVAVVNYKMPRLHTKKEVIENAKNIANMIVGMKQGLPGMDLVIFPEYSTMGIMYDRKEMFETATTIPGPETEIFAEACRKANTWGVFSLTGEQHEEHPHKNPYNTLVLINNKGEIVQKYRKIIPWCPIEGWYPGDTTYVTEGPKGIKISLIICDDGNYPEIWRDCAMKGAELIVRCQGYMYPAKEQQIMMAKTMAWANNVYVAVANATGFDGVYSYFGHSAIIGFDGRTLGECGEEENGIQYAEISLSQIRDFRQNAQSQNHLFKLLHRGYTGIIQSGEGDKGVAECPFDFYRTWVMDAEKARENVEKITRTTIGTAECPIEGIPHEGKEKEASV

SEQ ID NO: 43 - protein, 346 aa, Pseudomonas aeruginosa PAO1 [sequence omitted]

SEQ ID NO: 44 - protein, 340 aa, Methylophilus methylotrophus
MIHGDISSSQDTVGVAVVNYKMPRLHTKAEILANCRNIADMVVNMKAGLPGMDLVIFPEYSTHGIMYDSQEMYDNATTVPGPETDIFAEACRKAKVWGVFSITGEQHEEHPKKAPYNTLILMNDQGEIVQKYRKIMPWVPIEGWYPGKETFISEGPKGLKVSLIICDDGNYPEIWRDCAMKGAELIVRCQGYMYPAKEQQILISKAMAFANNTYVAVSNAAGFDGVYSYFGHSAIIGFDGRTLGECGEEENGVQYAALSKHLIRDFRKHGQSENHLFKLLHRGYTGMLNSGDGDQGVATCPYSFYSKWVQDPAAARDMVESFTRTTLGTKEAPIAGLPNE